European Patent Application EP 4 223 778 A1, published August 9, 2023. Title: Anti-claudin18.2 and cd3 bispecific antibody and use thereof. Applicant: INNOVENT BIOLOGICS (SUZHOU) CO., LTD. The sequence listing filed with the application follows.

SEQUENCE LISTING (42 sequences)

SEQ ID NO: 1 - protein, 10 aa, Artificial
  synthetic
GFTFSSYVMS

SEQ ID NO: 2 - protein, 17 aa, Artificial
  synthetic
TISHSGGSTYYADSVKG

SEQ ID NO: 3 - protein, 13 aa, Artificial
  synthetic
DAPYYDILTGYRY

SEQ ID NO: 4 - protein, 122 aa, Artificial
  synthetic
EVQLLDSGGGLVQPGGSLRLSCAASGFTFSSYVMSWVRQAPGKGLNWVSTISHSGGSTYYADSVKGRFTISRDNSKNTLYLQMNSLRAEDTAVYYCAIDAPYYDILTGYRYWGQGTLVTVSS

SEQ ID NO: 5 - protein, 330 aa, Artificial
  synthetic
ASTKGPSVFPLAPSSKSTSGGTAALGCLVKDYFPEPVTVSWNSGALTSGVHTFPAVLQSSGLYSLSSVVTVPSSSLGTQTYICNVNHKPSNTKVDKKAEPKSCDKTHTCPPCPAPELLGGPSVFLFPPKPKDTLMISRTPEVTCVVVDVSHEDPEVKFNWYVDGVEVHNAKTKPREEQYNSTYRVVSVLTVLHQDWLNGKEYKCKVSNKALPAPIEKTISKAKGQPREPQVYTLPPSRDELTKNQVSLTCLVKGFYPSDIAVEWESNGQPENNYKTTPPVLDSDGSFFLYSKLTVDKSRWQQGNVFSCSVMHEALHNHYTQKSLSLSPGK

SEQ ID NO: 6 - protein, 11 aa, Artificial
  synthetic
RASQSISSWLA

SEQ ID NO: 7 - protein, 7 aa, Artificial
  synthetic
KASSLES

SEQ ID NO: 8 - protein, 9 aa, Artificial
  synthetic
QQYNSYSYT

SEQ ID NO: 9 - protein, 107 aa, Artificial
  synthetic
DIQMTQSPSTLSASVGDRVTITCRASQSISSWLAWYQQKPGKAPKLLIYKASSLESGVPSRFSGSGSGTEFTLTISSLQPDDFATYYCQQYNSYSYTFGQGTKLEIK

SEQ ID NO: 10 - protein, 107 aa, Artificial [sequence omitted]

SEQ ID NO: 11 - protein, 10 aa, Artificial
  synthetic
GYTFTSYWIN

SEQ ID NO: 12 - protein, 16 aa, Artificial
  synthetic
NIYPSDSYTNYNQKFK

SEQ ID NO: 13 - protein, 9 aa, Artificial
  synthetic
SWRGNSFDY

SEQ ID NO: 14 - protein, 118 aa, Artificial
  synthetic
QVQLQQPGAELVRPGASVKLSCKASGYTFTSYWINWVKQRPGQGLEWIGNIYPSDSYTNYNQKFKDKATLTVDKSSSTAYMQLSSPTSEDSAVYYCTRSWRGNSFDYWGQGTTLTVSS

SEQ ID NO: 15 - protein, 17 aa, Artificial
  synthetic
KSSQSLLNSGNQKNYLT

SEQ ID NO: 16 - protein, 7 aa, Artificial
  synthetic
WASTRES

SEQ ID NO: 17 - protein, 9 aa, Artificial
  synthetic
QNDYSYPFT

SEQ ID NO: 18 - protein, 113 aa, Artificial
  synthetic
DIVMTQSPSSLTVTAGEKVTMSCKSSQSLLNSGNQKNYLTWYQQKPGQPPKLLIYWASTRESGVPDRFTGSGSGTDFTLTISSVQAEDLAVYYCQNDYSYPFTFGSGTKLEIK

SEQ ID NO: 19 - protein, 10 aa, Artificial
  synthetic
GFTFNTYAMN

SEQ ID NO: 20 - protein, 19 aa, Artificial
  synthetic
RIRSKYNNYATYYADSVKD

SEQ ID NO: 21 - protein, 14 aa, Artificial
  synthetic
HGNFGQSYVSWFAY

SEQ ID NO: 22 - protein, 125 aa, Artificial
  synthetic
EVQLVESGGGLVQPGGSLKLSCAASGFTFNTYAMNWVRQASGKGLEWVGRIRSKYNNYATYYADSVKDRFTISRDDSKSTLYLQMNSLKTEDTAVYYCARHGNFGQSYVSWFAYWGQGTTVTVSS

SEQ ID NO: 23 - protein, 330 aa, Artificial
  synthetic
ASTKGPSVFPLAPSSKSTSGGTAALGCLVKDYFPEPVTVSWNSGALTSGVHTFPAVLQSSGLYSLSSVVTVPSSSLGTQTYICNVNHKPSNTKVDKKVEPKSCDKTHTCPPCPAPEAAGGPSVFLFPPKPKDTLMISRTPEVTCVVVDVSHEDPEVKFNWYVDGVEVHNAKTKPREEQYNSTYRVVSVLTVLHQDWLNGKEYKCKVSNKALPAPIEKTISKAKGQPREPQVYTLPPSREEMTKNQVSLTCLVKGFYPSDIAVEWESNGQPENNYKTTPPVLDSDGSFFLYSKLTVDKSRWQQGNVFSCSVMHEALHNHYTQKSLSLSPGK

SEQ ID NO: 24 - protein, 14 aa, Artificial
  synthetic
RSSTGAVTTSNYAN

SEQ ID NO: 25 - protein, 7 aa, Artificial
  synthetic
GTNKRAP

SEQ ID NO: 26 - protein, 9 aa, Artificial
  synthetic
ALWYSNLWV

SEQ ID NO: 27 - protein, 109 aa, Artificial
  synthetic
QAVVTQEPSLTVSPGGTVTLTCRSSTGAVTTSNYANWVQQKPGQAPRGLIGGTNKRAPGVPARFSGSLLGDKAALTLLGAQPEDEAEYYCALWYSNLWVFGQGTKLTVL

SEQ ID NO: 28 - protein, 106 aa, Artificial
  synthetic
GQPKAAPSVTLFPPSSEELQANKATLVCLISDFYPGAVTVAWKADSSPVKAGVETTTPSKQSNNKYAASSYLSLTPEQWKSHRSYSCQVTHEGSTVEKTVAPTECS

SEQ ID NO: 29 - protein, 14 aa, Artificial
  synthetic
HYNFGQSYVSWFAY

SEQ ID NO: 30 - protein, 125 aa, Artificial
  synthetic
EVQLVESGGGLVQPGGSLKLSCAASGFTFNTYAMNWVRQASGKGLEWVGRIRSKYNNYATYYADSVKDRFTISRDDSKSTLYLQMNSLKTEDTAVYYCARHYNFGQSYVSWFAYWGQGTTVTVSS

SEQ ID NO: 31 - protein, 19 aa, Artificial
  synthetic
RIRSKAGGYATYYADSVKD

SEQ ID NO: 32 - protein, 125 aa, Artificial
  synthetic
EVQLVESGGGLVQPGGSLKLSCAASGFTFNTYAMNWVRQASGKGLEWVGRIRSKAGGYATYYADSVKDRFTISRDDSKSTLYLQMNSLKTEDTAVYYCARHGNFGQSYVSWFAYWGQGTTVTVSS

SEQ ID NO: 33 - protein, 330 aa, Artificial
  synthetic
ASTKGPSVFPLAPSSKSTSGGTAALGCLVKDYFPEPVTVSWNSGALTSGVHTFPAVLQSSGLYSLSSVVTVPSSSLGTQTYICNVNHKPSNTKVDKKVEPKSCDKTHTCPPCPAPEAAGGPSVFLFPPKPKDTLMISRTPEVTCVVVDVSHEDPEVKFNWYVDGVEVHNAKTKPREEQYNSTYRVVSVLTVLHQDWLNGKEYKCKVSNKALPAPIEKTISKAKGQPREPQVYTLPPSRDELTKNQVSLWCLVKGFYPSDIAVEWESNGQPENNYKTTPPVLDSDGSFFLYSKLTVDKSRWQQGNVFSCSVMHEALHNHYTQKSLSLSPGK

SEQ ID NO: 34 - protein, 330 aa, Artificial
  synthetic
ASTKGPSVFPLAPSSKSTSGGTAALGCLVKDYFPEPVTVSWNSGALTSGVHTFPAVLQSSGLYSLSSVVTVPSSSLGTQTYICNVNHKPSNTKVDKKVEPKSCDKTHTCPPCPAPEAAGGPSVFLFPPKPKDTLMISRTPEVTCVVVDVSHEDPEVKFNWYVDGVEVHNAKTKPREEQYNSTYRVVSVLTVLHQDWLNGKEYKCKVSNKALPAPIEKTISKAKGQPREPQVYTLPPSRDELTKNQVSLSCAVKGFYPSDIAVEWESNGQPENNYKTTPPVLDSDGSFFLVSKLTVDKSRWQQGNVFSCSVMHEALHNHYTQKSLSLSPGK

SEQ ID NO: 35 - protein, 125 aa, Artificial
  synthetic
EVQLVESGGGLVQPKGSLKLSCAASGFTFNTYAMNWVRQAPGKGLEWVARIRSKYNNYATYYADSVKDRFTISRDDSQSILYLQMNNLKTEDTAMYYCVRHGNFGNSYVSWFAYWGQGTLVTVSS

SEQ ID NO: 36 - protein, 109 aa, Artificial
  synthetic
QAVVTQESALTTSPGETVTLTCRSSTGAVTTSNYANWVQEKPDHLFTGLIGGTNKRAPGVPARFSGSLIGDKAALTITGAQTEDEAIYFCALWYSNLWVFGGGTKLTVL

SEQ ID NO: 37 - protein, 452 aa, Artificial
  synthetic
EVQLLDSGGGLVQPGGSLRLSCAASGFTFSSYVMSWVRQAPGKGLNWVSTISHSGGSTYYADSVKGRFTISRDNSKNTLYLQMNSLRAEDTAVYYCAIDAPYYDILTGYRYWGQGTLVTVSSASTKGPSVFPLAPSSKSTSGGTAALGCLVKDYFPEPVTVSWNSGALTSGVHTFPAVLQSSGLYSLSSVVTVPSSSLGTQTYICNVNHKPSNTKVDKKVEPKSCDKTHTCPPCPAPEAAGGPSVFLFPPKPKDTLMISRTPEVTCVVVDVSHEDPEVKFNWYVDGVEVHNAKTKPREEQYNSTYRVVSVLTVLHQDWLNGKEYKCKVSNKALPAPIEKTISKAKGQPREPQVYTLPPSRDELTKNQVSLWCLVKGFYPSDIAVEWESNGQPENNYKTTPPVLDSDGSFFLYSKLTVDKSRWQQGNVFSCSVMHEALHNHYTQKSLSLSPGK

SEQ ID NO: 38 - protein, 214 aa, Artificial
  synthetic
DIQMTQSPSTLSASVGDRVTITCRASQSISSWLAWYQQKPGKAPKLLIYKASSLESGVPSRFSGSGSGTEFTLTISSLQPDDFATYYCQQYNSYSYTFGQGTKLEIKRTVAAPSVFIFPPSDEQLKSGTASVVCLLNNFYPREAKVQWKVDNALQSGNSQESVTEQDSKDSTYSLSSTLTLSKADYEKHKVYACEVTHQGLSSPVTKSFNRGEC

SEQ ID NO: 39 - protein, 455 aa, Artificial
  synthetic
EVQLVESGGGLVQPGGSLKLSCAASGFTFNTYAMNWVRQASGKGLEWVGRIRSKYNNYATYYADSVKDRFTISRDDSKSTLYLQMNSLKTEDTAVYYCARHGNFGQSYVSWFAYWGQGTTVTVSSASTKGPSVFPLAPSSKSTSGGTAALGCLVKDYFPEPVTVSWNSGALTSGVHTFPAVLQSSGLYSLSSVVTVPSSSLGTQTYICNVNHKPSNTKVDKKVEPKSCDKTHTCPPCPAPEAAGGPSVFLFPPKPKDTLMISRTPEVTCVVVDVSHEDPEVKFNWYVDGVEVHNAKTKPREEQYNSTYRVVSVLTVLHQDWLNGKEYKCKVSNKALPAPIEKTISKAKGQPREPQVYTLPPSRDELTKNQVSLSCAVKGFYPSDIAVEWESNGQPENNYKTTPPVLDSDGSFFLVSKLTVDKSRWQQGNVFSCSVMHEALHNHYTQKSLSLSPGK

SEQ ID NO: 40 - protein, 215 aa, Artificial
  synthetic
QAVVTQEPSLTVSPGGTVTLTCRSSTGAVTTSNYANWVQQKPGQAPRGLIGGTNKRAPGVPARFSGSLLGDKAALTLLGAQPEDEAEYYCALWYSNLWVFGQGTKLTVLGQPKAAPSVTLFPPSSEELQANKATLVCLISDFYPGAVTVAWKADSSPVKAGVETTTPSKQSNNKYAASSYLSLTPEQWKSHRSYSCQVTHEGSTVEKTVAPTECS

SEQ ID NO: 41 - protein, 455 aa, Artificial
  synthetic
EVQLVESGGGLVQPGGSLKLSCAASGFTFNTYAMNWVRQASGKGLEWVGRIRSKYNNYATYYADSVKDRFTISRDDSKSTLYLQMNSLKTEDTAVYYCARHYNFGQSYVSWFAYWGQGTTVTVSSASTKGPSVFPLAPSSKSTSGGTAALGCLVKDYFPEPVTVSWNSGALTSGVHTFPAVLQSSGLYSLSSVVTVPSSSLGTQTYICNVNHKPSNTKVDKKVEPKSCDKTHTCPPCPAPEAAGGPSVFLFPPKPKDTLMISRTPEVTCVVVDVSHEDPEVKFNWYVDGVEVHNAKTKPREEQYNSTYRVVSVLTVLHQDWLNGKEYKCKVSNKALPAPIEKTISKAKGQPREPQVYTLPPSRDELTKNQVSLSCAVKGFYPSDIAVEWESNGQPENNYKTTPPVLDSDGSFFLVSKLTVDKSRWQQGNVFSCSVMHEALHNHYTQKSLSLSPGK

SEQ ID NO: 42 - protein, 455 aa, Artificial
  synthetic
EVQLVESGGGLVQPGGSLKLSCAASGFTFNTYAMNWVRQASGKGLEWVGRIRSKAGGYATYYADSVKDRFTISRDDSKSTLYLQMNSLKTEDTAVYYCARHGNFGQSYVSWFAYWGQGTTVTVSSASTKGPSVFPLAPSSKSTSGGTAALGCLVKDYFPEPVTVSWNSGALTSGVHTFPAVLQSSGLYSLSSVVTVPSSSLGTQTYICNVNHKPSNTKVDKKVEPKSCDKTHTCPPCPAPEAAGGPSVFLFPPKPKDTLMISRTPEVTCVVVDVSHEDPEVKFNWYVDGVEVHNAKTKPREEQYNSTYRVVSVLTVLHQDWLNGKEYKCKVSNKALPAPIEKTISKAKGQPREPQVYTLPPSRDELTKNQVSLSCAVKGFYPSDIAVEWESNGQPENNYKTTPPVLDSDGSFFLVSKLTVDKSRWQQGNVFSCSVMHEALHNHYTQKSLSLSPGK